European Patent Specification EP 3 868 391 B1, published May 22, 2024. Title: Inhibitor of Inflammatory Conditions. Applicant: Compton Developments Ltd. The sequence listing filed with the application follows.

SEQUENCE LISTING (6 sequences)

SEQ ID NO: 1 - DNA, 20 bp, Homo sapiens
tgttcagctgtgccttcaac

SEQ ID NO: 2 - DNA, 20 bp, Homo sapiens
aaagcgcagaactgagggta

SEQ ID NO: 3 - DNA, 20 bp, Homo sapiens
ggacgctcagagacatggag

SEQ ID NO: 4 - DNA, 21 bp, Homo sapiens
tatgccacggtgtgtaccata

SEQ ID NO: 5 - DNA, 20 bp, Homo sapiens
tagcacgcacgacatctttc

SEQ ID NO: 6 - DNA, 20 bp, Homo sapiens
gaaggtcacgtagcccacat